European Patent Application EP 4 275 701 A1, published November 15, 2023. Title: CONDITIONING REGIMEN FOR CELL TRANSPLANT. Applicant: HANSA BIOPHARMA AB. The sequence listing filed with the application follows.

SEQUENCE LISTING (92 sequences)

SEQ ID NO: 1 - protein, 339 aa, Streptococcus pyogenes
MRKRCYSTSAAVLAAVTLFVLSVDRGVIADSFSANQEIRYSEVTPYHVTSVWTKGVTPPANFTQGEDVFHAPYVANQGWYDITKTFNGKDDLLCGAATAGNMLHWWFDQNKDQIKRYLEEHPEKQKINFNGEQMFDVKEAIDTKNHQLDSKLFEYFKEKAFPYLSTKHLGVFPDHVIDMFINGYRLSLTNHGPTPVKEGSKDPRGGIFDAVFTRGDQSKLLTSRHDFKEKNLKEISDLIKKELTEGKALGLSHTYANVRINHVINLWGADFDSNGNLKAIYVTDSDSNASIGMKKYFVGVNSAGKVAISAKEIKEDNIGAQVLGLFTLSTGQDSWNQTN

SEQ ID NO: 2 - protein, 310 aa, Streptococcus pyogenes
DSFSANQEIRYSEVTPYHVTSVWTKGVTPPANFTQGEDVFHAPYVANQGWYDITKTFNGKDDLLCGAATAGNMLHWWFDQNKDQIKRYLEEHPEKQKINFNGEQMFDVKEAIDTKNHQLDSKLFEYFKEKAFPYLSTKHLGVFPDHVIDMFINGYRLSLTNHGPTPVKEGSKDPRGGIFDAVFTRGDQSKLLTSRHDFKEKNLKEISDLIKKELTEGKALGLSHTYANVRINHVINLWGADFDSNGNLKAIYVTDSDSNASIGMKKYFVGVNSAGKVAISAKEIKEDNIGAQVLGLFTLSTGQDSWNQTN

SEQ ID NO: 3 - protein, 349 aa, Streptococcus pyogenes
MKTIAYPNKPHSLSAGLLTAIAIFSLASSNITYADDYQRNATEAYAKEVPHQITSVWTKGVTPLTPEQFRYNNEDVIHAPYLAHQGWYDITKAFDGKDNLLCGAATAGNMLHWWFDQNKTEIEAYLSKHPEKQKIIFNNQELFDLKAAIDTKDSQTNSQLFNYFRDKAFPNLSARQLGVMPDLVLDMFINGYYLNVFKTQSTDVNRPYQDKDKRGGIFDAVFTRGDQTTLLTARHDLKNKGLNDISTIIKQELTEGRALALSHTYANVSISHVINLWGADFNAEGNLEAIYVTDSDANASIGMKKYFVGINAHGHVAISAKKIEGENIGAQVLGLFTLSSGKDIWQKLS

SEQ ID NO: 4 - protein, 315 aa, Streptococcus pyogenes
DDYQRNATEAYAKEVPHQITSVWTKGVTPLTPEQFRYNNEDVIHAPYLAHQGWYDITKAFDGKDNLLCGAATAGNMLHWWFDQNKTEIEAYLSKHPEKQKIIFNNQELFDLKAAIDTKDSQTNSQLFNYFRDKAFPNLSARQLGVMPDLVLDMFINGYYLNVFKTQSTDVNRPYQDKDKRGGIFDAVFTRGDQTTLLTARHDLKNKGLNDISTIIKQELTEGRALALSHTYANVSISHVINLWGADFNAEGNLEAIYVTDSDANASIGMKKYFVGINAHGHVAISAKKIEGENIGAQVLGLFTLSSGKDIWQKLS

SEQ ID NO: 5 - protein, 313 aa, Streptococcus pyogenes
DDYQRNATEAYAKEVPHQITSVWTKGVTPLTPEQFRYNNEDVFHAPYVANQGWYDITKAFDGKDNLLCGAATAGNMLHWWFDQNKDQIKRYLEEHPEKQKINFNGDNMFDVKKAIDTKNHQLDSKLFNYFKEKAFPGLSARRIGVFPDHVIDMFINGYRLSLTNHGPTPVKEGSKDPRGGIFDAVFTRGNQSKLLTSRHDFKNKNLNDISTIIKQELTKGKALGLSHTYANVSINHVINLWGADFNAEGNLEAIYVTDSDSNASIGMKKYFVGVNAHGHVAISAKKIEGENIGAQVLGLFTLSTGQDSWQKLS

SEQ ID NO: 6 - protein, 315 aa, Streptococcus pyogenes
DDYQRNATEAYAKEVPHQITSVWTKGVTPLTPEQFRYNNEDVIHAPYLANQGWYDITKAFDGKDNLLCGAATAGNMLHWWFDQNKTEIEAYLSKHPEKQKIIFRNQELFDLKEAIRTKDSQTNSQLFEYFRDKAFPYLSARQLGVMPDLVLDMFINGYYLNVFKTQSTDVKRPYQDKDKRGGIFDAVFTRGNQTTLLTARHDLKNKGLNDISTIIKEELTKGRALALSHTYANVSISHVINLWGADFNAEGNLEAIYVTDSDANASIGMKKYFVGINKHGHVAISAKKIEGENIGAQVLGLFTLSSGKDIWQKLN

SEQ ID NO: 7 - protein, 315 aa, Streptococcus pyogenes
DDYQRNATEAYAKEVPHQITSVWTKGVTPLTPEQFRYNNEDVIHAPYLAHQGWYDITKTFNGKDNLLCGAATAGNMLHWWFDQNKTEIEAYLSKHPEKQKIIFNNEELFDLKAAIDTKDSQTNSQLFNYFKEKAFPNLSTRQLGVMPDLVLDMFINGYYLNVFKTQSTDVNRPYQDKDKRGGIFDAVFTRGNQTTLLTARHDFKEKGLKDISTIIKQELTEGRALALSHTYANVSISHVINLWGADFDAEGNLKAIYVTDSDANASIGMKKYFVGINAHGKVAISAKKIEGENIGAQVLGLFTLSSGKDIWQQLS

SEQ ID NO: 8 - protein, 315 aa, Streptococcus pyogenes
DSFSANQEIRYSEVTPYHVTSVWTKGVTPLTPEQFRYNNEDVIHAPYLAHQGWYDITKAFDGKDNLLCGAATAGNMLHWWFDQNKTEIEAYLSKHPEKQKIIFNNQELFDLKAAIDTKDSQTNSQLFNYFRDKAFPNLSARQLGVMPDLVLDMFINGYYLNVFKTQSTDVNRPYQDKDKRGGIFDAVFTRGDQTTLLTARHDLKNKGLNDISTIIKQELTEGRALALSHTYANVSISHVINLWGADFNAEGNLEAIYVTDSDANASIGMKKYFVGINAHGHVAISAKKIEGENIGAQVLGLFTLSSGKDIWQKLS

SEQ ID NO: 9 - protein, 295 aa, Streptococcus pyogenes
SVWTKGVTPLTPEQFRYNNEDVIHAPYLAHQGWYDITKAFDGKDNLLCGAATAGNMLHWWFDQNKTEIEAYLSKHPEKQKIIFNNQELFDLKAAIDTKDSQTNSQLFNYFRDKAFPNLSARQLGVMPDLVLDMFINGYYLNVFKTQSTDVNRPYQDKDKRGGIFDAVFTRGDQTTLLTARHDLKNKGLNDISTIIKQELTEGRALALSHTYANVSISHVINLWGADFNAEGNLEAIYVTDSDANASIGMKKYFVGINAHGHVAISAKKIEGENIGAQVLGLFTLSSGKDIWQKLS

SEQ ID NO: 10 - protein, 314 aa, Streptococcus pyogenes
DDYQRNATEAYAKEVPHQITSVWTKGVTPLTPEQFTQGEDVIHAPYLAHQGWYDITKAFDGKDNLLCGAATAGNMLHWWFDQNKTEIEAYLSKHPEKQKIIFNNQELFDLKAAIDTKDSQTNSQLFNYFRDKAFPNLSARQLGVMPDLVLDMFINGYYLNVFKTQSTDVNRPYQDKDKRGGIFDAVFTRGDQTTLLTARHDLKNKGLNDISTIIKQELTEGRALALSHTYANVSISHVINLWGADFNAEGNLEAIYVTDSDANASIGMKKYFVGINAHGHVAISAKKIEGENIGAQVLGLFTLSSGKDIWQKLS

SEQ ID NO: 11 - protein, 312 aa, Streptococcus pyogenes
DDYQRNATEAYAKEVPHQITSVWTKGVTPPEQFTQGEDVIHAPYLAHQGWYDITKAFDGKDNLLCGAATAGNMLHWWFDQNKTEIEAYLSKHPEKQKIIFNNQELFDLKAAIDTKDSQTNSQLFNYFRDKAFPNLSARQLGVMPDLVLDMFINGYYLNVFKTQSTDVNRPYQDKDKRGGIFDAVFTRGDQTTLLTARHDLKNKGLNDISTIIKQELTEGRALALSHTYANVSISHVINLWGADFNAEGNLEAIYVTDSDANASIGMKKYFVGINAHGHVAISAKKIEGENIGAQVLGLFTLSSGKDIWQKLS

SEQ ID NO: 12 - protein, 313 aa, Streptococcus pyogenes
DDYQRNATEAYAKEVPHQITSVWTKGVTPPEQFRYNNEDVIHAPYLAHQGWYDITKAFDGKDNLLCGAATAGNMLHWWFDQNKTEIEAYLSKHPEKQKIIFNNQELFDLKAAIDTKDSQTNSQLFNYFRDKAFPNLSARQLGVMPDLVLDMFINGYYLNVFKTQSTDVNRPYQDKDKRGGIFDAVFTRGDQTTLLTARHDLKNKGLNDISTIIKQELTEGRALALSHTYANVSISHVINLWGADFNAEGNLEAIYVTDSDANASIGMKKYFVGINAHGHVAISAKKIEGENIGAQVLGLFTLSSGKDIWQKLS

SEQ ID NO: 13 - protein, 312 aa, Streptococcus pyogenes
DDYQRNATEAYAKEVPHQITSVWTKGVTPPEQFTQGEDVIHAPYLAHQGWYDITKAFDGKDNLLCGAATAGNMLHWWFDQNKTEIEAYLSKHPEKQKIIINNQELFDLKAAIDTKDSQTNSQLFNYFRDKAFPNLSARQLGVMPDLVLDMFINGYYLNVFKTQSTDVNRPYQDKDKRGGIFDAVFTRGDQTTLLTARHDLKNKGLNDISTIIKQELTEGRALALSHTYANVSISHVINLWGADFNAEGNLEAIYVTDSDANASIGMKKYFVGINAHGHVAISAKKIEGENIGAQVLGLFTLSSGKDIWQKLS

SEQ ID NO: 14 - protein, 312 aa, Streptococcus pyogenes
DDYQRNATEAYAKEVPHQITSVWTKGVTPPEQFTQGEDVIHAPYLAHQGWYDITKAFDGKDNLLCGAATAGNMLHWWFDQNKTEIEAYLSKHPEKQKIIFRNQELFDLKAAIDTKDSQTNSQLFNYFRDKAFPNLSARQLGVMPDLVLDMFINGYYLNVFKTQSTDVNRPYQDKDKRGGIFDAVFTRGDQTTLLTARHDLKNKGLNDISTIIKQELTEGRALALSHTYANVSISHVINLWGADFNAEGNLEAIYVTDSDANASIGMKKYFVGINAHGHVAISAKKIEGENIGAQVLGLFTLSSGKDIWQKLS

SEQ ID NO: 15 - protein, 312 aa, Streptococcus pyogenes
DDYQRNATEAYAKEVPHQITSVWTKGVTPPEQFTQGEDVIHAPYLAHQGWYDITKAFDGKDNLLCGAATAGNMLHWWFDQNKTEIEAYLSKHPEKQKIIIRNQELFDLKAAIDTKDSQTNSQLFNYFRDKAFPNLSARQLGVMPDLVLDMFINGYYLNVFKTQSTDVNRPYQDKDKRGGIFDAVFTRGDQTTLLTARHDLKNKGLNDISTIIKQELTEGRALALSHTYANVSISHVINLWGADFNAEGNLEAIYVTDSDANASIGMKKYFVGINAHGHVAISAKKIEGENIGAQVLGLFTLSSGKDIWQKLS

SEQ ID NO: 16 - protein, 312 aa, Streptococcus pyogenes
DDYQRNATEAYAKEVPHQITSVWTKGVTPPEQFTQGEDVIHAPYLANQGWYDITKAFDGKDNLLCGAATAGNMLHWWFDQNKTEIEAYLSKHPEKQKIIFRNQELFDLKEAIRTKDSQTNSQLFEYFRDKAFPYLSARQLGVMPDLVLDMFINGYYLNVFKTQSTDVKRPYQDKDKRGGIFDAVFTRGNQTTLLTARHDLKNKGLNDISTIIKEELTKGRALALSHTYANVSISHVINLWGADFNAEGNLEAIYVTDSDANASIGMKKYFVGINKHGHVAISAKKIEGENIGAQVLGLFTLSSGKDIWQKLN

SEQ ID NO: 17 - protein, 292 aa, Streptococcus pyogenes
SVWTKGVTPPEQFTQGEDVIHAPYLAHQGWYDITKAFDGKDNLLCGAATAGNMLHWWFDQNKTEIEAYLSKHPEKQKIIFRNQELFDLKAAIDTKDSQTNSQLFNYFRDKAFPNLSARQLGVMPDLVLDMFINGYYLNVFKTQSTDVNRPYQDKDKRGGIFDAVFTRGNQTTLLTARHDLKNKGLNDISTIIKQELTEGRALALSHTYANVSISHVINLWGADFNAEGNLEAIYVTDSDANASIGMKKYFVGINAHGHVAISAKKIEGENIGAQVLGLFTLSSGKDIWQKLS

SEQ ID NO: 18 - protein, 312 aa, Streptococcus pyogenes
DDYQRNATEAYAKEVPHQITSVWTKGVTPPEQFTQGEDVIHAPYLAHQGWYDITKAFDGADNLLCGAATAGNMLHWWFDQNKTEIEAYLSKHPEKQKIIFRNQELFDLKAAIDTKDSQTNSQLFNYFRDKAFPNLSARQLGVMPDLVLDMFINGYYLNVFKTQSTDVNRPYQDKDKRGGIFDAVFTRGNQTTLLTARHDLKNKGLNDISTIIKQELTEGRALALSHTYANVSISHVINLWGADFNAEGNLEAIYVTDSDANASIGMKKYFVGINAHGHVAISAKKIEGENIGAQVLGLFTLSSGKDIWQKLS

SEQ ID NO: 19 - protein, 292 aa, Streptococcus pyogenes
SVWTKGVTPPEQFTQGEDVIHAPYLAHQGWYDITKAFDGADNLLCGAATAGNMLHWWFDQNKTEIEAYLSKHPEKQKIIFRNQELFDLKAAIDTKDSQTNSQLFNYFRDKAFPNLSARQLGVMPDLVLDMFINGYYLNVFKTQSTDVNRPYQDKDKRGGIFDAVFTRGNQTTLLTARHDLKNKGLNDISTIIKQELTEGRALALSHTYANVSISHVINLWGADFNAEGNLEAIYVTDSDANASIGMKKYFVGINAHGHVAISAKKIEGENIGAQVLGLFTLSSGKDIWQKLS

SEQ ID NO: 20 - protein, 312 aa, Streptococcus pyogenes
DDYQRNATEAYAKEVPHQITSVWTKGVTPPEQFTQGEDVIHAPYLAHQGWYDITKAFDGKDNLLCGAATAGNMLHWWFDQNKTEIEAYLSKHPEKQKIIFRNQELFDLKAAIDTKDSQTNSQLFNYFRDKAFPNLSARQLGVMPDLVLDMFINGYYLNVFKTQSTDVNRPYQDKDKRGGIFDAVFTRGNQTTLLTARHDLKNKGLNDISTIIKQELTEGRALALSHTYANVSISHVINLWGADFNAEGNLEAIYVTDSDANASIGMKKYFVGINAHGHVAISAKKIEGENIGAQVLGLFTLSSGKDIWQKLS

SEQ ID NO: 21 - protein, 312 aa, Streptococcus pyogenes
DDYQRNATEAYAKEVPHQITSVWTKGVTPLTPEQFTQGEDVFHAPYVANQGWYDITKAFDGKDNLLCGAATAGNMLHWWFDQNKDQIKRYLEEHPEKQKINFNGENMFDVKKAIDTKNHQLDSKLFNYFKEKAFPYLSAKHLGVFPDHVIDMFINGYRLSLTNHGPTPVKEGSKDPRGGIFDAVFTRGNQSKLLTSRHDFKNKNLNDISTIIKQELTKGKALGLSHTYANVRINHVINLWGADFNAEGNLEAIYVTDSDSNASIGMKKYFVGVNAHGHVAISAKKIEGENIGAQVLGLFTLSTGQDSWQKLS

SEQ ID NO: 22 - protein, 312 aa, Streptococcus pyogenes
DDYQRNATEAYAKEVPHQITSVWTKGVTPLTPEQFTQGEDVFHAPYVANQGWYDITKAFDGKDNLLCGAATAGNMLHWWFDQNKDQIKRYLEEHPEKQKINFRGENMFDVKEAIRTKNHQLDSKLFEYFKEKAFPYLSAKHLGVFPDHVIDMFINGYRLSLTNHGPTPVKKGSKDPRGGIFDAVFTRGNQSKLLTSRHDFKNKNLNDISTIIKSELTNGKALGLSHTYANVRINHVINLWGADFNAEGNLEAIYVTDSDSNASIGMKKYFVGVNKHGHVAISAKKIEGENIGAQVLGLFTLSTGQDSWQKLN

SEQ ID NO: 23 - protein, 312 aa, Streptococcus pyogenes
DDYQRNATEAYAKEVPHQITSVWTKGVTPLTPEQFTQGEDVFHAPYVANQGWYDITKTFNGKDDLLCGAATAGNMLHWWFDQNKDQIKRYLEEHPEKQKINFNGEQMFDVKEAIDTKNHQLDSKLFEYFKEKAFPYLSTKHLGVFPDHVIDMFINGYRLSLTNHGPTPVKEGSKDPRGGIFDAVFTRGNQSKLLTSRHDFKEKNLKEISDLIKQELTEGKALGLSHTYANVRINHVINLWGADFDAEGNLKAIYVTDSDSNASIGMKKYFVGVNAAGKVAISAKKIEGENIGAQVLGLFTLSTGQDSWNQTS

SEQ ID NO: 24 - protein, 312 aa, Streptococcus pyogenes
DDYQRNATEAYAKEVPHQITSVWTKGVTPLTPEQFTQGEDVFHAPYVANQGWYDITKTFNGKDDLLCGAATAGNMLHWWFDQNKDQIKRYLEEHPEKQKINFRGEQMFDVKEAIRTKNHQLDSKLFEYFKEKAFPYLSTKHLGVFPDHVIDMFINGYRLSLTNHGPTPVKKGSKDPRGGIFDAVFTRGNQSKLLTSRHDFKEKNLKEISDLIKEELTKGKALGLSHTYANVRINHVINLWGADFDAEGNLKAIYVTDSDSNASIGMKKYFVGVNKAGKVAISAKKIEGENIGAQVLGLFTLSTGQDSWNQTN

SEQ ID NO: 25 - protein, 310 aa, Streptococcus pyogenes
DDYQRNATEAYAKEVPHQITSVWTKGVTPPEQFTQGEDVIHAPYVANQGWYDITKAFDGKDNLLCGAATAGNMLHWWFDQNKDQIKRYLEEHPEKQKINFRGEQMFDVKKAIDTKNHQLDSKLFNYFKEKAFPGLSARRIGVFPDHVIDMFINGYRLSLTNHGPTPVKEGSKDPRGGIFDAVFTRGNQSKLLTSRHDFKNKNLNDISTIIKQELTKGKALGLSHTYANVSINHVINLWGADFNAEGNLEAIYVTDSDSNASIGMKKYFVGVNAHGHVAISAKKIEGENIGAQVLGLFTLSTGQDSWQKLS

SEQ ID NO: 26 - protein, 320 aa, Streptococcus pyogenes
MDSFSANQEIRYSEVTPYHVTSVWTKGVTPPANFTQGEDVFHAPYVANQGWYDITKTFNGKDDLLCGAATAGNMLHWWFDQNKDQIKRYLEEHPEKQKINFNGEQMFDVKEAIDTKNHQLDSKLFEYFKEKAFPYLSTKHLGVFPDHVIDMFINGYRLSLTNHGPTPVKEGSKDPRGGIFDAVFTRGDQSKLLTSRHDFKEKNLKEISDLIKKELTEGKALGLSHTYANVRINHVINLWGADFDSNGNLKAIYVTDSDSNASIGMKKYFVGVNSAGKVAISAKEIKEDNIGAQVLGLFTLSTGQDSWNQTNGGGHHHHHH

SEQ ID NO: 27 - protein, 325 aa, Streptococcus pyogenes
MDDYQRNATEAYAKEVPHQITSVWTKGVTPLTPEQFRYNNEDVIHAPYLAHQGWYDITKAFDGKDNLLCGAATAGNMLHWWFDQNKTEIEAYLSKHPEKQKIIFNNQELFDLKAAIDTKDSQTNSQLFNYFRDKAFPNLSARQLGVMPDLVLDMFINGYYLNVFKTQSTDVNRPYQDKDKRGGIFDAVFTRGDQTTLLTARHDLKNKGLNDISTIIKQELTEGRALALSHTYANVSISHVINLWGADFNAEGNLEAIYVTDSDANASIGMKKYFVGINAHGHVAISAKKIEGENIGAQVLGLFTLSSGKDIWQKLSGGGHHHHHH

SEQ ID NO: 28 - protein, 323 aa, Streptococcus pyogenes
MDDYQRNATEAYAKEVPHQITSVWTKGVTPLTPEQFRYNNEDVFHAPYVANQGWYDITKAFDGKDNLLCGAATAGNMLHWWFDQNKDQIKRYLEEHPEKQKINFNGDNMFDVKKAIDTKNHQLDSKLFNYFKEKAFPGLSARRIGVFPDHVIDMFINGYRLSLTNHGPTPVKEGSKDPRGGIFDAVFTRGNQSKLLTSRHDFKNKNLNDISTIIKQELTKGKALGLSHTYANVSINHVINLWGADFNAEGNLEAIYVTDSDSNASIGMKKYFVGVNAHGHVAISAKKIEGENIGAQVLGLFTLSTGQDSWQKLSGGGHHHHHH

SEQ ID NO: 29 - protein, 11 aa, Streptococcus pyogenes
PLTPEQFRYNN

SEQ ID NO: 30 - protein, 8 aa, Streptococcus pyogenes
PPANFTQG

SEQ ID NO: 31 - protein, 20 aa, Streptococcus pyogenes
DDYQRNATEAYAKEVPHQIT

SEQ ID NO: 32 - protein, 20 aa, Streptococcus pyogenes
DSFSANQEIRYSEVTPYHVT

SEQ ID NO: 33 - DNA, 963 bp, Streptococcus pyogenes
atggatagtttttctgctaatcaagagattagatattcggaagtaacaccttatcacgttacttccgtttggaccaaaggagttactcctccagcaaacttcactcaaggtgaagatgtttttcacgctccttatgttgctaaccaaggatggtatgatattaccaaaacattcaatggaaaagacgatcttctttgcggggctgccacagcagggaatatgcttcactggtggttcgatcaaaacaaagaccaaattaaacgttatttggaagagcatccagaaaagcaaaaaataaacttcaatggcgaacagatgtttgacgtaaaagaagctatcgacactaaaaaccaccagctagatagtaaattatttgaatattttaaagaaaaagctttcccttatctatctactaaacacctaggagttttccctgatcatgtaattgatatgttcattaacggctaccgccttagtctaactaaccacggtccaacgccagtaaaagaaggtagtaaagatccccgaggtggtatttttgacgccgtatttacaagaggtgatcaaagtaagctattgacaagtcgtcatgattttaaagaaaaaaatctcaaagaaatcagtgatctcattaagaaagagttaaccgaaggcaaggctctaggcctatcacacacctacgctaacgtacgcatcaaccatgttataaacctgtggggagctgactttgattctaacgggaaccttaaagctatttatgtaacagactctgatagtaatgcatctattggtatgaagaaatactttgttggtgttaattccgctggaaaagtagctatttctgctaaagaaataaaagaagataatataggtgctcaagtactagggttatttacactttcaacagggcaagatagttggaatcagaccaatggcggtggccatcatcaccatcaccactaa

SEQ ID NO: 34 - DNA, 978 bp, Streptococcus pyogenes
atggacgattaccaaaggaatgctacggaagcttatgccaaagaagtaccacatcagatcacttctgtatggaccaaaggtgttacaccactaacacccgagcagtttcgatataataacgaagatgtgatccatgcgccatatcttgctcatcaaggctggtacgatatcaccaaggccttcgatgggaaggataatctcttgtgtggcgcagcaacggcaggtaatatgctgcattggtggtttgatcaaaataaaacagagattgaagcctatttaagtaaacaccctgaaaagcaaaaaatcatttttaacaaccaagagctatttgatttgaaagctgctatcgataccaaggacagtcaaaccaatagtcagctttttaattattttagagataaagcctttccaaatctatcagcacgtcaactcggggttatgcctgatcttgttctagatatgtttatcaatggttactacttaaatgtgtttaaaacacagtctactgatgtcaatcgaccttatcaggacaaggacaaacgaggtggtattttcgatgctgttttcaccagaggagatcagacaacgctcttgacagctcgtcatgatttaaaaaataaaggactaaatgacatcagcaccattatcaagcaagaactgactgaaggaagagcccttgctttatcacatacctacgccaatgttagcattagccatgtgattaacttgtggggagctgattttaatgctgaaggaaaccttgaggccatctatgtcacagactcagatgctaatgcgtctattggtatgaaaaaatattttgtcggcattaatgctcatggacatgtcgccatttctgccaagaaaatagaaggagaaaacattggcgctcaagtattaggcttatttacgctttccagtggcaaggacatttggcagaaactgagcggcggtggccatcatcaccatcaccactaa

SEQ ID NO: 35 - DNA, 972 bp, Streptococcus pyogenes
atggatgattatcagcgcaacgcgaccgaagcgtatgcgaaagaagtgccgcatcagattaccagcgtgtggaccaaaggcgtgaccccgctgaccccggaacagtttcgctataacaacgaagatgtgtttcatgcgccgtatgtggcgaaccagggctggtatgatattaccaaagcgtttgatggcaaagataacctgctgtgcggcgcggcgaccgcgggcaacatgctgcattggtggtttgatcagaacaaagatcagattaaacgctatctggaagaacatccggaaaaacagaaaattaactttaacggcgataacatgtttgatgtgaaaaaagcgattgataccaaaaaccatcagctggatagcaaactgtttaactattttaaagaaaaagcgtttccgggcctgagcgcgcgccgcattggcgtgtttccggatcatgtgattgatatgtttattaacggctatcgcctgagcctgaccaaccatggcccgaccccggtgaaagaaggcagcaaagatccgcgcggcggcatttttgatgcggtgtttacccgcggcaaccagagcaaactgctgaccagccgccatgattttaaaaacaaaaacctgaacgatattagcaccattattaaacaggaactgaccaaaggcaaagcgctgggcctgagccatacctatgcgaacgtgagcattaaccatgtgattaacctgtggggcgcggattttaacgcggaaggcaacctggaagcgatttatgtgaccgatagcgatagcaacgcgagcattggcatgaaaaaatattttgtgggcgtgaacgcgcatggccatgtggcgattagcgcgaaaaaaattgaaggcgaaaacattggcgcgcaggtgctgggcctgtttaccctgagcaccggccaggatagctggcagaaactgagcggcggtggccatcatcaccatcaccactaa

SEQ ID NO: 36 - DNA, 978 bp, Streptococcus pyogenes
atggatgattatcagcgcaacgcgaccgaagcgtatgcgaaagaagtgccgcatcagattaccagcgtgtggaccaaaggcgtgaccccgctgaccccggaacagtttcgctataacaacgaagatgtgattcatgcgccgtatctggcgaaccagggctggtatgatattaccaaagcgtttgatggcaaagataacctgctgtgcggcgcggcgaccgcgggcaacatgctgcattggtggtttgatcagaacaaaaccgaaattgaagcgtatctgagcaaacatccggaaaaacagaaaattatttttcgcaaccaggaactgtttgatctgaaagaagcgattcgcaccaaagatagccagaccaacagccagctgtttgaatattttcgcgataaagcgtttccgtatctgagcgcgcgccagctgggcgtgatgccggatctggtgctggatatgtttattaacggctattatctgaacgtgtttaaaacccagagcaccgatgtgaaacgcccgtatcaggataaagataaacgcggcggcatttttgatgcggtgtttacccgcggcaaccagaccaccctgctgaccgcgcgccatgatctgaaaaacaaaggcctgaacgatattagcaccattattaaagaagaactgaccaaaggccgcgcgctggcgctgagccatacctatgcgaacgtgagcattagccatgtgattaacctgtggggcgcggattttaacgcggaaggcaacctggaagcgatttatgtgaccgatagcgatgcgaacgcgagcattggcatgaaaaaatattttgtgggcattaacaaacatggccatgtggcgattagcgcgaaaaaaattgaaggcgaaaacattggcgcgcaggtgctgggcctgtttaccctgagcagcggcaaagatatttggcagaaactgaacggcggtggccatcatcaccatcaccactaa

SEQ ID NO: 37 - DNA, 978 bp, Streptococcus pyogenes
atggatgattatcagcgcaacgcgaccgaagcgtatgcgaaagaagtgccgcatcagattaccagcgtgtggaccaaaggcgtgaccccgctgaccccggaacagtttcgctataacaacgaagatgtgattcatgcgccgtatctggcgcatcagggctggtatgatattaccaaaacctttaacggcaaagataacctgctgtgcggcgcggcgaccgcgggcaacatgctgcattggtggtttgatcagaacaaaaccgaaattgaagcgtatctgagcaaacatccggaaaaacagaaaattatttttaacaacgaagaactgtttgatctgaaagcggcgattgataccaaagatagccagaccaacagccagctgtttaactattttaaagaaaaagcgtttccgaacctgagcacccgccagctgggcgtgatgccggatctggtgctggatatgtttattaacggctattatctgaacgtgtttaaaacccagagcaccgatgtgaaccgcccgtatcaggataaagataaacgcggcggcatttttgatgcggtgtttacccgcggcaaccagaccaccctgctgaccgcgcgccatgattttaaagaaaaaggcctgaaagatattagcaccattattaaacaggaactgaccgaaggccgcgcgctggcgctgagccatacctatgcgaacgtgagcattagccatgtgattaacctgtggggcgcggattttgatgcggaaggcaacctgaaagcgatttatgtgaccgatagcgatgcgaacgcgagcattggcatgaaaaaatattttgtgggcattaacgcgcatggcaaagtggcgattagcgcgaaaaaaattgaaggcgaaaacattggcgcgcaggtgctgggcctgtttaccctgagcagcggcaaagatatttggcagcagctgagcggcggtggccatcatcaccatcaccactaa

SEQ ID NO: 38 - DNA, 978 bp, Streptococcus pyogenes
atggatagctttagcgcgaaccaggaaattcgctatagcgaagtgaccccgtatcatgtgaccagcgtgtggaccaaaggcgtgaccccgctgaccccggaacagtttcgctataacaacgaagatgtgattcatgcgccgtatctggcgcatcagggctggtatgatattaccaaagcgtttgatggcaaagataacctgctgtgcggcgcggcgaccgcgggcaacatgctgcattggtggtttgatcagaacaaaaccgaaattgaagcgtatctgagcaaacatccggaaaaacagaaaattatttttaacaaccaggaactgtttgatctgaaagcggcgattgataccaaagatagccagaccaacagccagctgtttaactattttcgcgataaagcgtttccgaacctgagcgcgcgccagctgggcgtgatgccggatctggtgctggatatgtttattaacggctattatctgaacgtgtttaaaacccagagcaccgatgtgaaccgcccgtatcaggataaagataaacgcggcggcatttttgatgcggtgtttacccgcggcgatcagaccaccctgctgaccgcgcgccatgatctgaaaaacaaaggcctgaacgatattagcaccattattaaacaggaactgaccgaaggccgcgcgctggcgctgagccatacctatgcgaacgtgagcattagccatgtgattaacctgtggggcgcggattttaacgcggaaggcaacctggaagcgatttatgtgaccgatagcgatgcgaacgcgagcattggcatgaaaaaatattttgtgggcattaacgcgcatggccatgtggcgattagcgcgaaaaaaattgaaggcgaaaacattggcgcgcaggtgctgggcctgtttaccctgagcagcggcaaagatatttggcagaaactgagcggcggtggccatcatcaccatcaccactaa

SEQ ID NO: 39 - DNA, 918 bp, Streptococcus pyogenes
atgagcgtgtggaccaaaggcgtgaccccgctgaccccggaacagtttcgctataacaacgaagatgtgattcatgcgccgtatctggcgcatcagggctggtatgatattaccaaagcgtttgatggcaaagataacctgctgtgcggcgcggcgaccgcgggcaacatgctgcattggtggtttgatcagaacaaaaccgaaattgaagcgtatctgagcaaacatccggaaaaacagaaaattatttttaacaaccaggaactgtttgatctgaaagcggcgattgataccaaagatagccagaccaacagccagctgtttaactattttcgcgataaagcgtttccgaacctgagcgcgcgccagctgggcgtgatgccggatctggtgctggatatgtttattaacggctattatctgaacgtgtttaaaacccagagcaccgatgtgaaccgcccgtatcaggataaagataaacgcggcggcatttttgatgcggtgtttacccgcggcgatcagaccaccctgctgaccgcgcgccatgatctgaaaaacaaaggcctgaacgatattagcaccattattaaacaggaactgaccgaaggccgcgcgctggcgctgagccatacctatgcgaacgtgagcattagccatgtgattaacctgtggggcgcggattttaacgcggaaggcaacctggaagcgatttatgtgaccgatagcgatgcgaacgcgagcattggcatgaaaaaatattttgtgggcattaacgcgcatggccatgtggcgattagcgcgaaaaaaattgaaggcgaaaacattggcgcgcaggtgctgggcctgtttaccctgagcagcggcaaagatatttggcagaaactgagcggcggtggccatcatcaccatcaccactaa

SEQ ID NO: 40 - DNA, 975 bp, Streptococcus pyogenes
atggacgattaccaaaggaatgctacggaagcttatgccaaagaagtaccacatcagatcacttctgtatggaccaaaggtgttacaccactaacacccgagcagtttactcaaggtgaagatgtgatccatgcgccatatcttgctcatcaaggctggtacgatatcaccaaggccttcgatgggaaggataatctcttgtgtggcgcagcaacggcaggtaatatgctgcattggtggtttgatcaaaataaaacagagattgaagcctatttaagtaaacaccctgaaaagcaaaaaatcatttttaacaaccaagagctatttgatttgaaagctgctatcgataccaaggacagtcaaaccaatagtcagctttttaattattttagagataaagcctttccaaatctatcagcacgtcaactcggggttatgcctgatcttgttctagatatgtttatcaatggttactacttaaatgtgtttaaaacacagtctactgatgtcaatcgaccttatcaggacaaggacaaacgaggtggtattttcgatgctgttttcaccagaggagatcagacaacgctcttgacagctcgtcatgatttaaaaaataaaggactaaatgacatcagcaccattatcaagcaagaactgactgaaggaagagcccttgctttatcacatacctacgccaatgttagcattagccatgtgattaacttgtggggagctgattttaatgctgaaggaaaccttgaggccatctatgtcacagactcagatgctaatgcgtctattggtatgaaaaaatattttgtcggcattaatgctcatggacatgtcgccatttctgccaagaaaatagaaggagaaaacattggcgctcaagtattaggcttatttacgctttccagtggcaaggacatttggcagaaactgagcggcggtggccatcatcaccatcaccactaa

SEQ ID NO: 41 - DNA, 969 bp, Streptococcus pyogenes
atggacgattaccaaaggaatgctacggaagcttatgccaaagaagtaccacatcagatcacttctgtatggaccaaaggtgttacaccacccgagcagtttactcaaggtgaagatgtgatccatgcgccatatcttgctcatcaaggctggtacgatatcaccaaggccttcgatgggaaggataatctcttgtgtggcgcagcaacggcaggtaatatgctgcattggtggtttgatcaaaataaaacagagattgaagcctatttaagtaaacaccctgaaaagcaaaaaatcatttttaacaaccaagagctatttgatttgaaagctgctatcgataccaaggacagtcaaaccaatagtcagctttttaattattttagagataaagcctttccaaatctatcagcacgtcaactcggggttatgcctgatcttgttctagatatgtttatcaatggttactacttaaatgtgtttaaaacacagtctactgatgtcaatcgaccttatcaggacaaggacaaacgaggtggtattttcgatgctgttttcaccagaggagatcagacaacgctcttgacagctcgtcatgatttaaaaaataaaggactaaatgacatcagcaccattatcaagcaagaactgactgaaggaagagcccttgctttatcacatacctacgccaatgttagcattagccatgtgattaacttgtggggagctgattttaatgctgaaggaaaccttgaggccatctatgtcacagactcagatgctaatgcgtctattggtatgaaaaaatattttgtcggcattaatgctcatggacatgtcgccatttctgccaagaaaatagaaggagaaaacattggcgctcaagtattaggcttatttacgctttccagtggcaaggacatttggcagaaactgagcggcggtggccatcatcaccatcaccactaa

SEQ ID NO: 42 - DNA, 972 bp, Streptococcus pyogenes
atggacgattaccaaaggaatgctacggaagcttatgccaaagaagtaccacatcagatcacttctgtatggaccaaaggtgttacaccacccgagcagtttcgatataataacgaagatgtgatccatgcgccatatcttgctcatcaaggctggtacgatatcaccaaggccttcgatgggaaggataatctcttgtgtggcgcagcaacggcaggtaatatgctgcattggtggtttgatcaaaataaaacagagattgaagcctatttaagtaaacaccctgaaaagcaaaaaatcatttttaacaaccaagagctatttgatttgaaagctgctatcgataccaaggacagtcaaaccaatagtcagctttttaattattttagagataaagcctttccaaatctatcagcacgtcaactcggggttatgcctgatcttgttctagatatgtttatcaatggttactacttaaatgtgtttaaaacacagtctactgatgtcaatcgaccttatcaggacaaggacaaacgaggtggtattttcgatgctgttttcaccagaggagatcagacaacgctcttgacagctcgtcatgatttaaaaaataaaggactaaatgacatcagcaccattatcaagcaagaactgactgaaggaagagcccttgctttatcacatacctacgccaatgttagcattagccatgtgattaacttgtggggagctgattttaatgctgaaggaaaccttgaggccatctatgtcacagactcagatgctaatgcgtctattggtatgaaaaaatattttgtcggcattaatgctcatggacatgtcgccatttctgccaagaaaatagaaggagaaaacattggcgctcaagtattaggcttatttacgctttccagtggcaaggacatttggcagaaactgagcggcggtggccatcatcaccatcaccactaa

SEQ ID NO: 43 - DNA, 969 bp, Streptococcus pyogenes
atggacgattaccaaaggaatgctacggaagcttatgccaaagaagtaccacatcagatcacttctgtatggaccaaaggtgttacaccacccgagcagtttactcaaggtgaagatgtgatccatgcgccatatcttgctcatcaaggctggtacgatatcaccaaggccttcgatgggaaggataatctcttgtgtggcgcagcaacggcaggtaatatgctgcattggtggtttgatcaaaataaaacagagattgaagcctatttaagtaaacaccctgaaaagcaaaaaatcattattaacaaccaagagctatttgatttgaaagctgctatcgataccaaggacagtcaaaccaatagtcagctttttaattattttagagataaagcctttccaaatctatcagcacgtcaactcggggttatgcctgatcttgttctagatatgtttatcaatggttactacttaaatgtgtttaaaacacagtctactgatgtcaatcgaccttatcaggacaaggacaaacgaggtggtattttcgatgctgttttcaccagaggagatcagacaacgctcttgacagctcgtcatgatttaaaaaataaaggactaaatgacatcagcaccattatcaagcaagaactgactgaaggaagagcccttgctttatcacatacctacgccaatgttagcattagccatgtgattaacttgtggggagctgattttaatgctgaaggaaaccttgaggccatctatgtcacagactcagatgctaatgcgtctattggtatgaaaaaatattttgtcggcattaatgctcatggacatgtcgccatttctgccaagaaaatagaaggagaaaacattggcgctcaagtattaggcttatttacgctttccagtggcaaggacatttggcagaaactgagcggcggtggccatcatcaccatcaccactaa

SEQ ID NO: 44 - DNA, 969 bp, Streptococcus pyogenes
atggacgattaccaaaggaatgctacggaagcttatgccaaagaagtaccacatcagatcacttctgtatggaccaaaggtgttacaccacccgagcagtttactcaaggtgaagatgtgatccatgcgccatatcttgctcatcaaggctggtacgatatcaccaaggccttcgatgggaaggataatctcttgtgtggcgcagcaacggcaggtaatatgctgcattggtggtttgatcaaaataaaacagagattgaagcctatttaagtaaacaccctgaaaagcaaaaaatcatttttcgtaaccaagagctatttgatttgaaagctgctatcgataccaaggacagtcaaaccaatagtcagctttttaattattttagagataaagcctttccaaatctatcagcacgtcaactcggggttatgcctgatcttgttctagatatgtttatcaatggttactacttaaatgtgtttaaaacacagtctactgatgtcaatcgaccttatcaggacaaggacaaacgaggtggtattttcgatgctgttttcaccagaggagatcagacaacgctcttgacagctcgtcatgatttaaaaaataaaggactaaatgacatcagcaccattatcaagcaagaactgactgaaggaagagcccttgctttatcacatacctacgccaatgttagcattagccatgtgattaacttgtggggagctgattttaatgctgaaggaaaccttgaggccatctatgtcacagactcagatgctaatgcgtctattggtatgaaaaaatattttgtcggcattaatgctcatggacatgtcgccatttctgccaagaaaatagaaggagaaaacattggcgctcaagtattaggcttatttacgctttccagtggcaaggacatttggcagaaactgagcggcggtggccatcatcaccatcaccactaa

SEQ ID NO: 45 - DNA, 969 bp, Streptococcus pyogenes
atggacgattaccaaaggaatgctacggaagcttatgccaaagaagtaccacatcagatcacttctgtatggaccaaaggtgttacaccacccgagcagtttactcaaggtgaagatgtgatccatgcgccatatcttgctcatcaaggctggtacgatatcaccaaggccttcgatgggaaggataatctcttgtgtggcgcagcaacggcaggtaatatgctgcattggtggtttgatcaaaataaaacagagattgaagcctatttaagtaaacaccctgaaaagcaaaaaatcattattcgtaaccaagagctatttgatttgaaagctgctatcgataccaaggacagtcaaaccaatagtcagctttttaattattttagagataaagcctttccaaatctatcagcacgtcaactcggggttatgcctgatcttgttctagatatgtttatcaatggttactacttaaatgtgtttaaaacacagtctactgatgtcaatcgaccttatcaggacaaggacaaacgaggtggtattttcgatgctgttttcaccagaggagatcagacaacgctcttgacagctcgtcatgatttaaaaaataaaggactaaatgacatcagcaccattatcaagcaagaactgactgaaggaagagcccttgctttatcacatacctacgccaatgttagcattagccatgtgattaacttgtggggagctgattttaatgctgaaggaaaccttgaggccatctatgtcacagactcagatgctaatgcgtctattggtatgaaaaaatattttgtcggcattaatgctcatggacatgtcgccatttctgccaagaaaatagaaggagaaaacattggcgctcaagtattaggcttatttacgctttccagtggcaaggacatttggcagaaactgagcggcggtggccatcatcaccatcaccactaa

SEQ ID NO: 46 - DNA, 969 bp, Streptococcus pyogenes
atggatgattatcagcgcaacgcgaccgaagcgtatgcgaaagaagtgccgcatcagattaccagcgtgtggaccaaaggcgtgaccccgccggaacagtttactcaaggtgaagatgtgattcatgcgccgtatctggcgaaccagggctggtatgatattaccaaagcgtttgatggcaaagataacctgctgtgcggcgcggcgaccgcgggcaacatgctgcattggtggtttgatcagaacaaaaccgaaattgaagcgtatctgagcaaacatccggaaaaacagaaaattatttttcgcaaccaggaactgtttgatctgaaagaagcgattcgcaccaaagatagccagaccaacagccagctgtttgaatattttcgcgataaagcgtttccgtatctgagcgcgcgccagctgggcgtgatgccggatctggtgctggatatgtttattaacggctattatctgaacgtgtttaaaacccagagcaccgatgtgaaacgcccgtatcaggataaagataaacgcggcggcatttttgatgcggtgtttacccgcggcaaccagaccaccctgctgaccgcgcgccatgatctgaaaaacaaaggcctgaacgatattagcaccattattaaagaagaactgaccaaaggccgcgcgctggcgctgagccatacctatgcgaacgtgagcattagccatgtgattaacctgtggggcgcggattttaacgcggaaggcaacctggaagcgatttatgtgaccgatagcgatgcgaacgcgagcattggcatgaaaaaatattttgtgggcattaacaaacatggccatgtggcgattagcgcgaaaaaaattgaaggcgaaaacattggcgcgcaggtgctgggcctgtttaccctgagcagcggcaaagatatttggcagaaactgaacggcggtggccatcatcaccatcaccactaa

SEQ ID NO: 47 - DNA, 909 bp, Streptococcus pyogenes
atgtctgtatggaccaaaggtgttacaccacccgagcagtttactcaaggtgaagatgtgatccatgcgccatatcttgctcatcaaggctggtacgatatcaccaaggccttcgatgggaaggataatctcttgtgtggcgcagcaacggcaggtaatatgctgcattggtggtttgatcaaaataaaacagagattgaagcctatttaagtaaacaccctgaaaagcaaaaaatcatttttcgtaaccaagagctatttgatttgaaagctgctatcgataccaaggacagtcaaaccaatagtcagctttttaattattttagagataaagcctttccaaatctatcagcacgtcaactcggggttatgcctgatcttgttctagatatgtttatcaatggttactacttaaatgtgtttaaaacacagtctactgatgtcaatcgaccttatcaggacaaggacaaacgaggtggtattttcgatgctgttttcaccagaggaaaccagacaacgctcttgacagctcgtcatgatttaaaaaataaaggactaaatgacatcagcaccattatcaagcaagaactgactgaaggaagagcccttgctttatcacatacctacgccaatgttagcattagccatgtgattaacttgtggggagctgattttaatgctgaaggaaaccttgaggccatctatgtcacagactcagatgctaatgcgtctattggtatgaaaaaatattttgtcggcattaatgctcatggacatgtcgccatttctgccaagaaaatagaaggagaaaacattggcgctcaagtattaggcttatttacgctttccagtggcaaggacatttggcagaaactgagcggcggtggccatcatcaccatcaccactaa

SEQ ID NO: 48 - DNA, 969 bp, Streptococcus pyogenes
atggacgattaccaaaggaatgctacggaagcttatgccaaagaagtaccacatcagatcacttctgtatggaccaaaggtgttacaccacccgagcagtttactcaaggtgaagatgtgatccatgcgccatatcttgctcatcaaggctggtacgatatcaccaaggccttcgatggggcggataatctcttgtgtggcgcagcaacggcaggtaatatgctgcattggtggtttgatcaaaataaaacagagattgaagcctatttaagtaaacaccctgaaaagcaaaaaatcatttttcgtaaccaagagctatttgatttgaaagctgctatcgataccaaggacagtcaaaccaatagtcagctttttaattattttagagataaagcctttccaaatctatcagcacgtcaactcggggttatgcctgatcttgttctagatatgtttatcaatggttactacttaaatgtgtttaaaacacagtctactgatgtcaatcgaccttatcaggacaaggacaaacgaggtggtattttcgatgctgttttcaccagaggaaatcagacaacgctcttgacagctcgtcatgatttaaaaaataaaggactaaatgacatcagcaccattatcaagcaagaactgactgaaggaagagcccttgctttatcacatacctacgccaatgttagcattagccatgtgattaacttgtggggagctgattttaatgctgaaggaaaccttgaggccatctatgtcacagactcagatgctaatgcgtctattggtatgaaaaaatattttgtcggcattaatgctcatggacatgtcgccatttctgccaagaaaatagaaggagaaaacattggcgctcaagtattaggcttatttacgctttccagtggcaaggacatttggcagaaactgagcggcggtggccatcatcaccatcaccactaa

SEQ ID NO: 49 - DNA, 909 bp, Streptococcus pyogenes
atgtctgtatggaccaaaggtgttacaccacccgagcagtttactcaaggtgaagatgtgatccatgcgccatatcttgctcatcaaggctggtacgatatcaccaaggccttcgatggggcggataatctcttgtgtggcgcagcaacggcaggtaatatgctgcattggtggtttgatcaaaataaaacagagattgaagcctatttaagtaaacaccctgaaaagcaaaaaatcatttttcgtaaccaagagctatttgatttgaaagctgctatcgataccaaggacagtcaaaccaatagtcagctttttaattattttagagataaagcctttccaaatctatcagcacgtcaactcggggttatgcctgatcttgttctagatatgtttatcaatggttactacttaaatgtgtttaaaacacagtctactgatgtcaatcgaccttatcaggacaaggacaaacgaggtggtattttcgatgctgttttcaccagaggaaatcagacaacgctcttgacagctcgtcatgatttaaaaaataaaggactaaatgacatcagcaccattatcaagcaagaactgactgaaggaagagcccttgctttatcacatacctacgccaatgttagcattagccatgtgattaacttgtggggagctgattttaatgctgaaggaaaccttgaggccatctatgtcacagactcagatgctaatgcgtctattggtatgaaaaaatattttgtcggcattaatgctcatggacatgtcgccatttctgccaagaaaatagaaggagaaaacattggcgctcaagtattaggcttatttacgctttccagtggcaaggacatttggcagaaactgagcggcggtggccatcatcaccatcaccactaa

SEQ ID NO: 50 - DNA, 969 bp, Streptococcus pyogenes
atggacgattaccaaaggaatgctacggaagcttatgccaaagaagtaccacatcagatcacttctgtatggaccaaaggtgttacaccacccgagcagtttactcaaggtgaagatgtgatccatgcgccatatcttgctcatcaaggctggtacgatatcaccaaggccttcgatgggaaggataatctcttgtgtggcgcagcaacggcaggtaatatgctgcattggtggtttgatcaaaataaaacagagattgaagcctatttaagtaaacaccctgaaaagcaaaaaatcatttttcgtaaccaagagctatttgatttgaaagctgctatcgataccaaggacagtcaaaccaatagtcagctttttaattattttagagataaagcctttccaaatctatcagcacgtcaactcggggttatgcctgatcttgttctagatatgtttatcaatggttactacttaaatgtgtttaaaacacagtctactgatgtcaatcgaccttatcaggacaaggacaaacgaggtggtattttcgatgctgttttcaccagaggaaaccagacaacgctcttgacagctcgtcatgatttaaaaaataaaggactaaatgacatcagcaccattatcaagcaagaactgactgaaggaagagcccttgctttatcacatacctacgccaatgttagcattagccatgtgattaacttgtggggagctgattttaatgctgaaggaaaccttgaggccatctatgtcacagactcagatgctaatgcgtctattggtatgaaaaaatattttgtcggcattaatgctcatggacatgtcgccatttctgccaagaaaatagaaggagaaaacattggcgctcaagtattaggcttatttacgctttccagtggcaaggacatttggcagaaactgagcggcggtggccatcatcaccatcaccactaa

SEQ ID NO: 51 - DNA, 969 bp, Streptococcus pyogenes
atggatgattatcagcgcaacgcgaccgaagcgtatgcgaaagaagtgccgcatcagattaccagcgtgtggaccaaaggcgtgaccccgctgaccccggaacagtttacccagggcgaagatgtgtttcatgcgccgtatgtggcgaaccagggctggtatgatattaccaaagcgtttgatggcaaagataacctgctgtgcggcgcggcgaccgcgggcaacatgctgcattggtggtttgatcagaacaaagatcagattaaacgctatctggaagaacatccggaaaaacagaaaattaactttaacggcgaaaacatgtttgatgtgaaaaaagcgattgataccaaaaaccatcagctggatagcaaactgtttaactattttaaagaaaaagcgtttccgtatctgagcgcgaaacatctgggcgtgtttccggatcatgtgattgatatgtttattaacggctatcgcctgagcctgaccaaccatggcccgaccccggtgaaagaaggcagcaaagatccgcgcggcggcatttttgatgcggtgtttacccgcggcaaccagagcaaactgctgaccagccgccatgattttaaaaacaaaaacctgaacgatattagcaccattattaaacaggaactgaccaaaggcaaagcgctgggcctgagccatacctatgcgaacgtgcgcattaaccatgtgattaacctgtggggcgcggattttaacgcggaaggcaacctggaagcgatttatgtgaccgatagcgatagcaacgcgagcattggcatgaaaaaatattttgtgggcgtgaacgcgcatggccatgtggcgattagcgcgaaaaaaattgaaggcgaaaacattggcgcgcaggtgctgggcctgtttaccctgagcaccggccaggatagctggcagaaactgagcggcggtggccatcatcaccatcaccactaa

SEQ ID NO: 52 - DNA, 969 bp, Streptococcus pyogenes
atggatgattatcagcgcaacgcgaccgaagcgtatgcgaaagaagtgccgcatcagattaccagcgtgtggaccaaaggcgtgaccccgctgaccccggaacagtttacccagggcgaagatgtgtttcatgcgccgtatgtggcgaaccagggctggtatgatattaccaaagcgtttgatggcaaagataacctgctgtgcggcgcggcgaccgcgggcaacatgctgcattggtggtttgatcagaacaaagatcagattaaacgctatctggaagaacatccggaaaaacagaaaattaactttcgcggcgaaaacatgtttgatgtgaaagaagcgattcgcaccaaaaaccatcagctggatagcaaactgtttgaatattttaaagaaaaagcgtttccgtatctgagcgcgaaacatctgggcgtgtttccggatcatgtgattgatatgtttattaacggctatcgcctgagcctgaccaaccatggcccgaccccggtgaaaaaaggcagcaaagatccgcgcggcggcatttttgatgcggtgtttacccgcggcaaccagagcaaactgctgaccagccgccatgattttaaaaacaaaaacctgaacgatattagcaccattattaaaagcgaactgaccaacggcaaagcgctgggcctgagccatacctatgcgaacgtgcgcattaaccatgtgattaacctgtggggcgcggattttaacgcggaaggcaacctggaagcgatttatgtgaccgatagcgatagcaacgcgagcattggcatgaaaaaatattttgtgggcgtgaacaaacatggccatgtggcgattagcgcgaaaaaaattgaaggcgaaaacattggcgcgcaggtgctgggcctgtttaccctgagcaccggccaggatagctggcagaaactgaacggcggtggccatcatcaccatcaccactaa

SEQ ID NO: 53 - DNA, 969 bp, Streptococcus pyogenes
atggatgattatcagcgcaacgcgaccgaagcgtatgcgaaagaagtgccgcatcagattaccagcgtgtggaccaaaggcgtgaccccgctgaccccggaacagtttacccagggcgaagatgtgtttcatgcgccgtatgtggcgaaccagggctggtatgatattaccaaaacctttaacggcaaagatgatctgctgtgcggcgcggcgaccgcgggcaacatgctgcattggtggtttgatcagaacaaagatcagattaaacgctatctggaagaacatccggaaaaacagaaaattaactttaacggcgaacagatgtttgatgtgaaagaagcgattgataccaaaaaccatcagctggatagcaaactgtttgaatattttaaagaaaaagcgtttccgtatctgagcaccaaacatctgggcgtgtttccggatcatgtgattgatatgtttattaacggctatcgcctgagcctgaccaaccatggcccgaccccggtgaaagaaggcagcaaagatccgcgcggcggcatttttgatgcggtgtttacccgcggcaaccagagcaaactgctgaccagccgccatgattttaaagaaaaaaacctgaaagaaattagcgatctgattaaacaggaactgaccgaaggcaaagcgctgggcctgagccatacctatgcgaacgtgcgcattaaccatgtgattaacctgtggggcgcggattttgatgcggaaggcaacctgaaagcgatttatgtgaccgatagcgatagcaacgcgagcattggcatgaaaaaatattttgtgggcgtgaacgcggcgggcaaagtggcgattagcgcgaaaaaaattgaaggcgaaaacattggcgcgcaggtgctgggcctgtttaccctgagcaccggccaggatagctggaaccagaccagcggcggtggccatcatcaccatcaccactaa

SEQ ID NO: 54 - DNA, 969 bp, Streptococcus pyogenes
atggatgattatcagcgcaacgcgaccgaagcgtatgcgaaagaagtgccgcatcagattaccagcgtgtggaccaaaggcgtgaccccgctgaccccggaacagtttacccagggcgaagatgtgtttcatgcgccgtatgtggcgaaccagggctggtatgatattaccaaaacctttaacggcaaagatgatctgctgtgcggcgcggcgaccgcgggcaacatgctgcattggtggtttgatcagaacaaagatcagattaaacgctatctggaagaacatccggaaaaacagaaaattaactttcgcggcgaacagatgtttgatgtgaaagaagcgattcgcaccaaaaaccatcagctggatagcaaactgtttgaatattttaaagaaaaagcgtttccgtatctgagcaccaaacatctgggcgtgtttccggatcatgtgattgatatgtttattaacggctatcgcctgagcctgaccaaccatggcccgaccccggtgaaaaaaggcagcaaagatccgcgcggcggcatttttgatgcggtgtttacccgcggcaaccagagcaaactgctgaccagccgccatgattttaaagaaaaaaacctgaaagaaattagcgatctgattaaagaagaactgaccaaaggcaaagcgctgggcctgagccatacctatgcgaacgtgcgcattaaccatgtgattaacctgtggggcgcggattttgatgcggaaggcaacctgaaagcgatttatgtgaccgatagcgatagcaacgcgagcattggcatgaaaaaatattttgtgggcgtgaacaaagcgggcaaagtggcgattagcgcgaaaaaaattgaaggcgaaaacattggcgcgcaggtgctgggcctgtttaccctgagcaccggccaggatagctggaaccagaccaacggcggtggccatcatcaccatcaccactaa

SEQ ID NO: 55 - DNA, 963 bp, Streptococcus pyogenes
atggatgattatcagcgcaacgcgaccgaagcgtatgcgaaagaagtgccgcatcagattaccagcgtgtggaccaaaggcgtgaccccgccggaacagtttactcaaggtgaagatgtgattcatgcgccgtatgtggcgaaccagggctggtatgatattaccaaagcgtttgatggcaaagataacctgctgtgcggcgcggcgaccgcgggcaacatgctgcattggtggtttgatcagaacaaagatcagattaaacgctatctggaagaacatccggaaaaacagaaaattaactttcgcggcgaacagatgtttgatgtgaaaaaagcgattgataccaaaaaccatcagctggatagcaaactgtttaactattttaaagaaaaagcgtttccgggcctgagcgcgcgccgcattggcgtgtttccggatcatgtgattgatatgtttattaacggctatcgcctgagcctgaccaaccatggcccgaccccggtgaaagaaggcagcaaagatccgcgcggcggcatttttgatgcggtgtttacccgcggcaaccagagcaaactgctgaccagccgccatgattttaaaaacaaaaacctgaacgatattagcaccattattaaacaggaactgaccaaaggcaaagcgctgggcctgagccatacctatgcgaacgtgagcattaaccatgtgattaacctgtggggcgcggattttaacgcggaaggcaacctggaagcgatttatgtgaccgatagcgatagcaacgcgagcattggcatgaaaaaatattttgtgggcgtgaacgcgcatggccatgtggcgattagcgcgaaaaaaattgaaggcgaaaacattggcgcgcaggtgctgggcctgtttaccctgagcaccggccaggatagctggcagaaactgagcggcggtggccatcatcaccatcaccactaa

SEQ ID NO: 56 - protein, 310 aa, Streptococcus pyogenes
DSFSANQEIRYSEVTPYHVTSVWTKGVTPPANFTQGEDVFHAPYVANQGWYDITKTFNGKDDLLCGAATAGNMLHWWFDQNKDQIKRYLEEHPEKQKINFRGEQMFDVKEAIDTKNHQLDSKLFEYFKEKAFPYLSTKHLGVFPDHVIDMFINGYRLSLTNHGPTPVKEGSKDPRGGIFDAVFTRGDQSKLLTSRHDFKEKNLKEISDLIKKELTEGKALGLSHTYANVRINHVINLWGADFDSNGNLKAIYVTDSDSNASIGMKKYFVGVNSAGKVAISAKEIKEDNIGAQVLGLFTLSTGQDSWNQTN

SEQ ID NO: 57 - protein, 310 aa, Streptococcus pyogenes
DSFSANQEIRYSEVTPYHVTSVWTKGVTPPANFTQGEDVFHAPYVANQGWYDITKTFNGKDDLLCGAATAGNMLHWWFDQNKDQIKRYLEEHPEKQKINFKGEQMFDVKEAIDTKNHQLDSKLFEYFKEKAFPYLSTKHLGVFPDHVIDMFINGYRLSLTNHGPTPVKRGSKDPRGGIFDAVFTRGNQSKLLTSRHDFKEKNLKEISDLIKKELTEGKALGLSHTYANVRINHVINLWGADFDSNGNLKAIYVTDSDSNASIGMKKYFVGVNSAGKVAISAKEIKEDNIGAQVLGLFTLSTGQDSWNQTN

SEQ ID NO: 58 - protein, 310 aa, Streptococcus pyogenes
DSFSANQEIRYSEVTPYHVTSVWTKGVTPPANFTQGEDVFHAPYVANQGWYDITKTFNGKDDLLCGAATAGNMLHWWFDQNKDQIKRYLEEHPEKQKINFRGEQMFDVKEAIDTKNHQLDSKLFEYFKEKAFPYLSTKHLGVFPDHVIDMFINGYRLSLTNHGPTPVKKGSKDPRGGIFDAVFTRGNQSKLLTSRHDFKEKNLKEISDLIKKELTEGKALGLSHTYANVRINHVINLWGADFDSNGNLKAIYVTDSDSNASIGMKKYFVGVNKAGKVAISAKEIKEDNIGAQVLGLFTLSTGQDSWNQTN

SEQ ID NO: 59 - protein, 310 aa, Streptococcus pyogenes
DSFSANQEIRYSEVTPYHVTSVWTKGVTPPANFTQGEDVFHAPYVANQGWYDITKTFNGKDDLLCGAATAGNMLHWWFDQNKDQIKRYLREHPEKQKINFNGEQMFDVKEAIDTKNHQLDSKLFEYFKEKAFPYLSTKHLGVFPDHVIDMFINGYRLSLTNHGPTPVKEGSKDPRGGIFDAVFTRGNQSKLLTSRHDFKEKNLKEISDLIKKELDEGKALGLSHTYANVRINHVINLWGADFDSNGNLKAIYVTDSDSNASIGMKKYFVGVNSAGKVAISAKEIKEDNIGAQVLGLFTLSTGQDSWNQTN

SEQ ID NO: 60 - protein, 310 aa, Streptococcus pyogenes
DSFSANQEIRYSEVTPYHVTSVWTKGVTPPANFTQGEDVFHAPYVANQGWYDITKTFNGKDDLLCGAATAGNMLHWWFDQNKDQIKRYLKEHPEKQKINFNGEQMFDVKEAIRTKNHQLDSKLFEYFKEKAFPYLSTKHLGVFPDHVIDMFINGYRLSLTNHGPTPVKEGSKDPRGGIFDAVFTRGNQSKLLTSRHDFKEKNLKEISDLIKKELEEGKALGLSHTYANVRINHVINLWGADFDSNGNLKAIYVTDSDSNASIGMKKYFVGVNKAGKVAISAKEIKEDNIGAQVLGLFTLSTGQDSWNQTN

SEQ ID NO: 61 - protein, 310 aa, Streptococcus pyogenes
DSFSANQEIRYSEVTPYHVTSVWTKGVTPPANFTQGEDVFHAPYVANQGWYDITKTFNGKDDLLCGAATAGNMLHWWFDQNKDQIERYLEEHPEKQKINFNGEQMFDVKEAIDTKNHQLDSKLFEYFKEKAFPYLSTKHLGVFPDHVIDMFINGYRLSLTNHGPTPVKEGSKDPRGGIFDAVFTRGNQSKLLTSRHDFKEKNLKEISDLIKEELTKGKALGLSHTYANVRINHVINLWGADFDSNGNLKAIYVTDSDSNASIGMKKYFVGVNSAGKVAISAKEIKEKNIGAQVLGLFTLSTGQKSWNQTN

SEQ ID NO: 62 - protein, 310 aa, Streptococcus pyogenes
DSFSANQEIRYSEVTPYHVTSVWTKGVTPPANFTQGEDVFHAPYVANQGWYDITKTFNGKDDLLCGAATAGNMLHWWFDQNKDQIKRYLKEHPEKQKINFRGEQMFDVKEAIRTKNHQLDSKLFEYFKEKAFPYLSTKHLGVFPDHVIDMFINGYRLSLTNHGPTPVKEGSKDPRGGIFDAVFTRGNQSKLLTSRHDFKEKNLKEISDLIKSELENGKALGLSHTYANVRINHVINLWGADFDSNGNLKAIYVTDSDSNASIGMKKYFVGVNKAGKVAISAKEIKEDNIGAQVLGLFTLSTGQDSWNQTN

SEQ ID NO: 63 - protein, 310 aa, Streptococcus pyogenes
DSFSANQEIRYSEVTPYHVTSVWTKGVTPPANFTQGEDVFHAPYVANQGWYDITKTFNGKDDLLCGAATAGNMLHWWFDQNKDQIKRYLKEHPEKQKINFRGEQMFDVKEAIRTKNHQLDSKLFEYFKEKAFPYLSTKHLGVFPDHVIDMFINGYRLSLTNHGPTPVKKGSKDPRGGIFDAVFTRGNQSKLLTSRHDFKEKNLKEISDLIKKELEEGKALGLSHTYANVRINHVINLWGADFDSNGNLKAIYVTDSDSNASIGMKKYFVGVNSAGKVAISAKEIKEDNIGAQVLGLFTLSTGQDSWNQTN

SEQ ID NO: 64 - protein, 310 aa, Streptococcus pyogenes
DSFSANQEIRYSEVTPYHVTSVWTKGVTPPANFTQGEDVFHAPYVANQGWYDITKTFNGKDDLLCGAATAGNMLHWWFDQNKDQIERYLEEHPEKQKINFRGEQMFDVKEAIDTKNHQLDSKLFEYFKEKAFPYLSTKHLGVFPDHVIDMFINGYRLSLTNHGPTPVKKGSKDPRGGIFDAVFTRGNQSKLLTSRHDFKEKNLKEISDLIKEELTKGKALGLSHTYANVRINHVINLWGADFDSNGNLKAIYVTDSDSNASIGMKKYFVGVNSAGKVAISAKEIKEDNIGAQVLGLFTLSTGQKSWNQTN

SEQ ID NO: 65 - protein, 306 aa, Streptococcus pyogenes
DSFSANQEIRYSEVTPYHVTSVWTKGVTPPANFTQGEDVFHAPYVANQGWYDITKTFNGKDDLLCGAATAGNMLHWWFDQNKDQIKRYLEEHPEKQKINFNGEQMFDVKEAIDTKNHQLDSKLFEYFKEKAFPYLSTKHLGVFPDHVIDMFINGYRLSLTNHGPTPVKEGSKDPRGGIFDAVFTRGDQSKLLTSRHDFKEKNLKEISDLIKKELTEGKALGLSHTYANVRINHVINLWGADFDSNGNLKAIYVTDSDSNASIGMKKYFVGVNSAGKVAISAKEIKEDNIGAQVLGLFTLSTGQDSW

SEQ ID NO: 66 - protein, 290 aa, Streptococcus pyogenes
SVWTKGVTPPANFTQGEDVFHAPYVANQGWYDITKTFNGKDDLLCGAATAGNMLHWWFDQNKDQIKRYLEEHPEKQKINFNGEQMFDVKEAIDTKNHQLDSKLFEYFKEKAFPYLSTKHLGVFPDHVIDMFINGYRLSLTNHGPTPVKEGSKDPRGGIFDAVFTRGDQSKLLTSRHDFKEKNLKEISDLIKKELTEGKALGLSHTYANVRINHVINLWGADFDSNGNLKAIYVTDSDSNASIGMKKYFVGVNSAGKVAISAKEIKEDNIGAQVLGLFTLSTGQDSWNQTN

SEQ ID NO: 67 - protein, 290 aa, Streptococcus pyogenes
SVWTKGVTPPANFTQGEDVFHAPYVANQGWYDITKTFNGKDDLLCGAATAGNMLHWWFDQNKDQIKRYLEEHPEKQKINFKGEQMFDVKEAIDTKNHQLDSKLFEYFKEKAFPYLSTKHLGVFPDHVIDMFINGYRLSLTNHGPTPVKEGSKDPRGGIFDAVFTRGNQSKLLTSRHDFKEKNLKEISDLIKKELTEGKALGLSHTYANVRINHVINLWGADFDSNGNLKAIYVTDSDSNASIGMKKYFVGVNSAGKVAISAKEIKEDNIGAQVLGLFTLSTGQDSWNQTN

SEQ ID NO: 68 - protein, 290 aa, Streptococcus pyogenes
SVWTKGVTPPANFTQGEDVFHAPYVANQGWYDITKTFNGKDDLLCGAATAGNMLHWWFDQNKDQIERYLEEHPEKQKINFKGEQMFDVKKAIDTKNHQLDSKLFEYFKEKAFPYLSTKHLGVFPDHVIDMFINGYRLSLTNHGPTPVKEGSKDPRGGIFDAVFTRGNQSKLLTSRHDFKEKNLKEISDLIKEELTKGKALGLSHTYANVRINHVINLWGADFDSNGNLKAIYVTDSDSNASIGMKKYFVGVNSAGKVAISAKEIKEDNIGAQVLGLFTLSTGQKSWNQTN

SEQ ID NO: 69 - protein, 319 aa, Streptococcus pyogenes
DDYQRNATEAYAKEVPHQITSVWTKGVTPPANFTQGEDVFHAPYVANQGWYDITKTFNGKDDLLCGAATAGNMLHWWFDQNKDQIERYLEEHPEKQKINFKGEQMFDVKKAIDTKNHQLDSKLFEYFKEKAFPYLSTKHLGVFPDHVIDMFINGYRLSLTNHGPTPVKEGSKDPRGGIFDAVFTRGNQSKLLTSRHDFKEKNLKEISDLIKEELTKGKALGLSHTYANVRINHVINLWGADFDSNGNLKAIYVTDSDSNASIGMKKYFVGVNSAGKVAISAKEIKEDNIGAQVLGLFTLSTGQKSWNQTNGGGHHHHHH

SEQ ID NO: 70 - protein, 4 aa, Streptococcus pyogenes
NQTN

SEQ ID NO: 71 - protein, 20 aa, Streptococcus pyogenes
DSFSANQEIRYSEVTPYHVT

SEQ ID NO: 72 - DNA, 963 bp, Streptococcus pyogenes; identical to SEQ ID NO: 33

SEQ ID NO: 73 - DNA, 963 bp, Streptococcus pyogenes
atggatagtttttctgctaatcaagagattagatattcggaagtaacaccttatcacgttacttccgtttggaccaaaggagttactcctccagcaaacttcactcaaggtgaagatgtttttcacgctccttatgttgctaaccaaggatggtatgatattaccaaaacattcaatggaaaagacgatcttctttgcggggctgccacagcagggaatatgcttcactggtggttcgatcaaaacaaagaccaaattaaacgttatttggaagagcatccagaaaagcaaaaaataaacttccgtggcgaacagatgtttgacgtaaaagaagctatcgacactaaaaaccaccagctagatagtaaattatttgaatattttaaagaaaaagctttcccttatctatctactaaacacctaggagttttccctgatcatgtaattgatatgttcattaacggctaccgccttagtctaactaaccacggtccaacgccagtaaaagaaggtagtaaagatccccgaggtggtatttttgacgccgtatttacaagaggtgatcaaagtaagctattgacaagtcgtcatgattttaaagaaaaaaatctcaaagaaatcagtgatctcattaagaaagagttaaccgaaggcaaggctctaggcctatcacacacctacgctaacgtacgcatcaaccatgttataaacctgtggggagctgactttgattctaacgggaaccttaaagctatttatgtaacagactctgatagtaatgcatctattggtatgaagaaatactttgttggtgttaattccgctggaaaagtagctatttctgctaaagaaataaaagaagataatataggtgctcaagtactagggttatttacactttcaacagggcaagatagttggaatcagaccaatggcggtggccatcatcaccatcaccactaa

SEQ ID NO: 74 - DNA, 963 bp, Streptococcus pyogenes
atggatagtttttctgctaatcaagagattagatattcggaagtaacaccttatcacgttacttccgtttggaccaaaggagttactcctccagcaaacttcactcaaggtgaagatgtttttcacgctccttatgttgctaaccaaggatggtatgatattaccaaaacattcaatggaaaagacgatcttctttgcggggctgccacagcagggaatatgcttcactggtggttcgatcaaaacaaagaccaaattaaacgttatttggaagagcatccagaaaagcaaaaaataaacttcaaaggcgaacagatgtttgacgtaaaagaagctatcgacactaaaaaccaccagctagatagtaaattatttgaatattttaaagaaaaagctttcccttatctatctactaaacacctaggagttttccctgatcatgtaattgatatgttcattaacggctaccgccttagtctaactaaccacggtccaacgccagtaaaacgtggtagtaaagatccccgaggtggtatttttgacgccgtatttacaagaggtaaccaaagtaagctattgacaagtcgtcatgattttaaagaaaaaaatctcaaagaaatcagtgatctcattaagaaagagttaaccgaaggcaaggctctaggcctatcacacacctacgctaacgtacgcatcaaccatgttataaacctgtggggagctgactttgattctaacgggaaccttaaagctatttatgtaacagactctgatagtaatgcatctattggtatgaagaaatactttgttggtgttaattccgctggaaaagtagctatttctgctaaagaaataaaagaagataatataggtgctcaagtactagggttatttacactttcaacagggcaagatagttggaatcagaccaatggcggtggccatcatcaccatcaccactaa

SEQ ID NO: 75 - DNA, 963 bp, Streptococcus pyogenes
atggatagtttttctgctaatcaagagattagatattcggaagtaacaccttatcacgttacttccgtttggaccaaaggagttactcctccagcaaacttcactcaaggtgaagatgtttttcacgctccttatgttgctaaccaaggatggtatgatattaccaaaacattcaatggaaaagacgatcttctttgcggggctgccacagcagggaatatgcttcactggtggttcgatcaaaacaaagaccaaattaaacgttatttggaagagcatccagaaaagcaaaaaataaacttccgtggcgaacagatgtttgacgtaaaagaagctatcgacactaaaaaccaccagctagatagtaaattatttgaatattttaaagaaaaagctttcccttatctatctactaaacacctaggagttttccctgatcatgtaattgatatgttcattaacggctaccgccttagtctaactaaccacggtccaacgccagtaaaaaaaggtagtaaagatccccgaggtggtatttttgacgccgtatttacaagaggtaaccaaagtaagctattgacaagtcgtcatgattttaaagaaaaaaatctcaaagaaatcagtgatctcattaagaaagagttaaccgaaggcaaggctctaggcctatcacacacctacgctaacgtacgcatcaaccatgttataaacctgtggggagctgactttgattctaacgggaaccttaaagctatttatgtaacagactctgatagtaatgcatctattggtatgaagaaatactttgttggtgttaataaagctggaaaagtagctatttctgctaaagaaataaaagaagataatataggtgctcaagtactagggttatttacactttcaacagggcaagatagttggaatcagaccaatggcggtggccatcatcaccatcaccactaa

SEQ ID NO: 76 - DNA, 963 bp, Streptococcus pyogenes
atggatagtttttctgctaatcaagagattagatattcggaagtaacaccttatcacgttacttccgtttggaccaaaggagttactcctccagcaaacttcactcaaggtgaagatgtttttcacgctccttatgttgctaaccaaggatggtatgatattaccaaaacattcaatggaaaagacgatcttctttgcggggctgccacagcagggaatatgcttcactggtggttcgatcaaaacaaagaccaaattaaacgttatttgcgtgagcatccagaaaagcaaaaaataaacttcaatggcgaacagatgtttgacgtaaaagaagctatcgacactaaaaaccaccagctagatagtaaattatttgaatattttaaagaaaaagctttcccttatctatctactaaacacctaggagttttccctgatcatgtaattgatatgttcattaacggctaccgccttagtctaactaaccacggtccaacgccagtaaaagaaggtagtaaagatccccgaggtggtatttttgacgccgtatttacaagaggtaaccaaagtaagctattgacaagtcgtcatgattttaaagaaaaaaatctcaaagaaatcagtgatctcattaagaaagagttagatgaaggcaaggctctaggcctatcacacacctacgctaacgtacgcatcaaccatgttataaacctgtggggagctgactttgattctaacgggaaccttaaagctatttatgtaacagactctgatagtaatgcatctattggtatgaagaaatactttgttggtgttaattccgctggaaaagtagctatttctgctaaagaaataaaagaagataatataggtgctcaagtactagggttatttacactttcaacagggcaagatagttggaatcagaccaatggcggtggccatcatcaccatcaccactaa

SEQ ID NO: 77 - DNA, 963 bp, Streptococcus pyogenes
atggatagtttttctgctaatcaagagattagatattcggaagtaacaccttatcacgttacttccgtttggaccaaaggagttactcctccagcaaacttcactcaaggtgaagatgtttttcacgctccttatgttgctaaccaaggatggtatgatattaccaaaacattcaatggaaaagacgatcttctttgcggggctgccacagcagggaatatgcttcactggtggttcgatcaaaacaaagaccaaattaaacgttatttgaaagagcatccagaaaagcaaaaaataaacttcaatggcgaacagatgtttgacgtaaaagaagctatccgtactaaaaaccaccagctagatagtaaattatttgaatattttaaagaaaaagctttcccttatctatctactaaacacctaggagttttccctgatcatgtaattgatatgttcattaacggctaccgccttagtctaactaaccacggtccaacgccagtaaaagaaggtagtaaagatccccgaggtggtatttttgacgccgtatttacaagaggtaaccaaagtaagctattgacaagtcgtcatgattttaaagaaaaaaatctcaaagaaatcagtgatctcattaagaaagagttagaagaaggcaaggctctaggcctatcacacacctacgctaacgtacgcatcaaccatgttataaacctgtggggagctgactttgattctaacgggaaccttaaagctatttatgtaacagactctgatagtaatgcatctattggtatgaagaaatactttgttggtgttaataaagctggaaaagtagctatttctgctaaagaaataaaagaagataatataggtgctcaagtactagggttatttacactttcaacagggcaagatagttggaatcagaccaatggcggtggccatcatcaccatcaccactaa

SEQ ID NO: 78 - DNA, 963 bp, Streptococcus pyogenes
atggatagtttttctgctaatcaagagattagatattcggaagtaacaccttatcacgttacttccgtttggaccaaaggagttactcctccagcaaacttcactcaaggtgaagatgtttttcacgctccttatgttgctaaccaaggatggtatgatattaccaaaacattcaatggaaaagacgatcttctttgcggggctgccacagcagggaatatgcttcactggtggttcgatcaaaacaaagaccaaattgaacgttatttggaagagcatccagaaaagcaaaaaataaacttcaatggcgaacagatgtttgacgtaaaagaagctatcgacactaaaaaccaccagctagatagtaaattatttgaatattttaaagaaaaagctttcccttatctatctactaaacacctaggagttttccctgatcatgtaattgatatgttcattaacggctaccgccttagtctaactaaccacggtccaacgccagtaaaagaaggtagtaaagatccccgaggtggtatttttgacgccgtatttacaagaggtaaccaaagtaagctattgacaagtcgtcatgattttaaagaaaaaaatctcaaagaaatcagtgatctcattaaggaagagttaaccaaaggcaaggctctaggcctatcacacacctacgctaacgtacgcatcaaccatgttataaacctgtggggagctgactttgattctaacgggaaccttaaagctatttatgtaacagactctgatagtaatgcatctattggtatgaagaaatactttgttggtgttaattccgctggaaaagtagctatttctgctaaagaaataaaagaaaaaaatataggtgctcaagtactagggttatttacactttcaacagggcaaaaaagttggaatcagaccaatggcggtggccatcatcaccatcaccactaa

SEQ ID NO: 79 - DNA, 963 bp, Streptococcus pyogenes
atggatagtttttctgctaatcaagagattagatattcggaagtaacaccttatcacgttacttccgtttggaccaaaggagttactcctccagcaaacttcactcaaggtgaagatgtttttcacgctccttatgttgctaaccaaggatggtatgatattaccaaaacattcaatggaaaagacgatcttctttgcggggctgccacagcagggaatatgcttcactggtggttcgatcaaaacaaagaccaaattaaacgttatttgaaagagcatccagaaaagcaaaaaataaacttccgtggcgaacagatgtttgacgtaaaagaagctatccgtactaaaaaccaccagctagatagtaaattatttgaatattttaaagaaaaagctttcccttatctatctactaaacacctaggagttttccctgatcatgtaattgatatgttcattaacggctaccgccttagtctaactaaccacggtccaacgccagtaaaagaaggtagtaaagatccccgaggtggtatttttgacgccgtatttacaagaggtaaccaaagtaagctattgacaagtcgtcatgattttaaagaaaaaaatctcaaagaaatcagtgatctcattaagagtgagttagaaaacggcaaggctctaggcctatcacacacctacgctaacgtacgcatcaaccatgttataaacctgtggggagctgactttgattctaacgggaaccttaaagctatttatgtaacagactctgatagtaatgcatctattggtatgaagaaatactttgttggtgttaataaagctggaaaagtagctatttctgctaaagaaataaaagaagataatataggtgctcaagtactagggttatttacactttcaacagggcaagatagttggaatcagaccaatggcggtggccatcatcaccatcaccactaa

SEQ ID NO: 80 - DNA, 963 bp, Streptococcus pyogenes
atggatagtttttctgctaatcaagagattagatattcggaagtaacaccttatcacgttacttccgtttggaccaaaggagttactcctccagcaaacttcactcaaggtgaagatgtttttcacgctccttatgttgctaaccaaggatggtatgatattaccaaaacattcaatggaaaagacgatcttctttgcggggctgccacagcagggaatatgcttcactggtggttcgatcaaaacaaagaccaaattaaacgttatttgaaagagcatccagaaaagcaaaaaataaacttccgtggcgaacagatgtttgacgtaaaagaagctatccgtactaaaaaccaccagctagatagtaaattatttgaatattttaaagaaaaagctttcccttatctatctactaaacacctaggagttttccctgatcatgtaattgatatgttcattaacggctaccgccttagtctaactaaccacggtccaacgccagtaaaaaaaggtagtaaagatccccgaggtggtatttttgacgccgtatttacaagaggtaaccaaagtaagctattgacaagtcgtcatgattttaaagaaaaaaatctcaaagaaatcagtgatctcattaagaaagagttagaagaaggcaaggctctaggcctatcacacacctacgctaacgtacgcatcaaccatgttataaacctgtggggagctgactttgattctaacgggaaccttaaagctatttatgtaacagactctgatagtaatgcatctattggtatgaagaaatactttgttggtgttaattccgctggaaaagtagctatttctgctaaagaaataaaagaagataatataggtgctcaagtactagggttatttacactttcaacagggcaagatagttggaatcagaccaatggcggtggccatcatcaccatcaccactaa

SEQ ID NO: 81 - DNA, 963 bp, Streptococcus pyogenes
atggatagtttttctgctaatcaagagattagatattcggaagtaacaccttatcacgttacttccgtttggaccaaaggagttactcctccagcaaacttcactcaaggtgaagatgtttttcacgctccttatgttgctaaccaaggatggtatgatattaccaaaacattcaatggaaaagacgatcttctttgcggggctgccacagcagggaatatgcttcactggtggttcgatcaaaacaaagaccaaattgaacgttatttggaagagcatccagaaaagcaaaaaataaacttccgtggcgaacagatgtttgacgtaaaagaagctatcgacactaaaaaccaccagctagatagtaaattatttgaatattttaaagaaaaagctttcccttatctatctactaaacacctaggagttttccctgatcatgtaattgatatgttcattaacggctaccgccttagtctaactaaccacggtccaacgccagtaaaaaaaggtagtaaagatccccgaggtggtatttttgacgccgtatttacaagaggtaaccaaagtaagctattgacaagtcgtcatgattttaaagaaaaaaatctcaaagaaatcagtgatctcattaaggaagagttaaccaaaggcaaggctctaggcctatcacacacctacgctaacgtacgcatcaaccatgttataaacctgtggggagctgactttgattctaacgggaaccttaaagctatttatgtaacagactctgatagtaatgcatctattggtatgaagaaatactttgttggtgttaattccgctggaaaagtagctatttctgctaaagaaataaaagaagataatataggtgctcaagtactagggttatttacactttcaacagggcaaaaaagttggaatcagaccaatggcggtggccatcatcaccatcaccactaa

SEQ ID NO: 82 - DNA, 957 bp, Streptococcus pyogenes
atggatagtttttctgctaatcaagagattagatattcggaagtaacaccttatcacgttacttccgtttggaccaaaggagttactcctccagcaaacttcactcaaggtgaagatgtttttcacgctccttatgttgctaaccaaggatggtatgatattaccaaaacattcaatggaaaagacgatcttctttgcggggctgccacagcagggaatatgcttcactggtggttcgatcaaaacaaagaccaaattaaacgttatttggaagagcatccagaaaagcaaaaaataaacttcaatggcgaacagatgtttgacgtaaaagaagctatcgacactaaaaaccaccagctagatagtaaattatttgaatattttaaagaaaaagctttcccttatctatctactaaacacctaggagttttccctgatcatgtaattgatatgttcattaacggctaccgccttagtctaactaaccacggtccaacgccagtaaaagaaggtagtaaagatccccgaggtggtatttttgacgccgtatttacaagaggtgatcaaagtaagctattgacaagtcgtcatgattttaaagaaaaaaatctcaaagaaatcagtgatctcattaagaaagagttaaccgaaggcaaggctctaggcctatcacacacctacgctaacgtacgcatcaaccatgttataaacctgtggggagctgactttgattctaacgggaaccttaaagctatttatgtaacagactctgatagtaatgcatctattggtatgaagaaatactttgttggtgttaattccgctggaaaagtagctatttctgctaaagaaataaaagaagataatataggtgctcaagtactagggttatttacactttcaacagggcaagatagttggggtggcggcggtggccatcatcaccatcaccactaa

SEQ ID NO: 83 - DNA, 903 bp, Streptococcus pyogenes
atgtccgtttggaccaaaggagttactcctccagcaaacttcactcaaggtgaagatgtttttcacgctccttatgttgctaaccaaggatggtatgatattaccaaaacattcaatggaaaagacgatcttctttgcggggctgccacagcagggaatatgcttcactggtggttcgatcaaaacaaagaccaaattaaacgttatttggaagagcatccagaaaagcaaaaaataaacttcaatggcgaacagatgtttgacgtaaaagaagctatcgacactaaaaaccaccagctagatagtaaattatttgaatattttaaagaaaaagctttcccttatctatctactaaacacctaggagttttccctgatcatgtaattgatatgttcattaacggctaccgccttagtctaactaaccacggtccaacgccagtaaaagaaggtagtaaagatccccgaggtggtatttttgacgccgtatttacaagaggtgatcaaagtaagctattgacaagtcgtcatgattttaaagaaaaaaatctcaaagaaatcagtgatctcattaagaaagagttaaccgaaggcaaggctctaggcctatcacacacctacgctaacgtacgcatcaaccatgttataaacctgtggggagctgactttgattctaacgggaaccttaaagctatttatgtaacagactctgatagtaatgcatctattggtatgaagaaatactttgttggtgttaattccgctggaaaagtagctatttctgctaaagaaataaaagaagataatataggtgctcaagtactagggttatttacactttcaacagggcaagatagttggaatcagaccaatggcggtggccatcatcaccatcaccactaa

SEQ ID NO: 84 - DNA, 903 bp, Streptococcus pyogenes
atgtccgtttggaccaaaggagttactcctccagcaaacttcactcaaggtgaagatgtttttcacgctccttatgttgctaaccaaggatggtatgatattaccaaaacattcaatggaaaagacgatcttctttgcggggctgccacagcagggaatatgcttcactggtggttcgatcaaaacaaagaccaaattaaacgttatttggaagagcatccagaaaagcaaaaaataaacttcaaaggcgaacagatgtttgacgtaaaagaagctatcgacactaaaaaccaccagctagatagtaaattatttgaatattttaaagaaaaagctttcccttatctatctactaaacacctaggagttttccctgatcatgtaattgatatgttcattaacggctaccgccttagtctaactaaccacggtccaacgccagtaaaagaaggtagtaaagatccccgaggtggtatttttgacgccgtatttacaagaggtaaccaaagtaagctattgacaagtcgtcatgattttaaagaaaaaaatctcaaagaaatcagtgatctcattaagaaagagttaaccgaaggcaaggctctaggcctatcacacacctacgctaacgtacgcatcaaccatgttataaacctgtggggagctgactttgattctaacgggaaccttaaagctatttatgtaacagactctgatagtaatgcatctattggtatgaagaaatactttgttggtgttaattccgctggaaaagtagctatttctgctaaagaaataaaagaagataatataggtgctcaagtactagggttatttacactttcaacagggcaagatagttggaatcagaccaatggcggtggccatcatcaccatcaccactaa

SEQ ID NO: 85 - DNA, 903 bp, Streptococcus pyogenes
atgtccgtttggaccaaaggagttactcctccagcaaacttcactcaaggtgaagatgtttttcacgctccttatgttgctaaccaaggatggtatgatattaccaaaacattcaatggaaaagacgatcttctttgcggggctgccacagcagggaatatgcttcactggtggttcgatcaaaacaaagaccaaattgaacgttatttggaagagcatccagaaaagcaaaaaataaacttcaaaggcgaacagatgtttgacgtaaaaaaagctatcgacactaaaaaccaccagctagatagtaaattatttgaatattttaaagaaaaagctttcccttatctatctactaaacacctaggagttttccctgatcatgtaattgatatgttcattaacggctaccgccttagtctaactaaccacggtccaacgccagtaaaagaaggtagtaaagatccccgaggtggtatttttgacgccgtatttacaagaggtaaccaaagtaagctattgacaagtcgtcatgattttaaagaaaaaaatctcaaagaaatcagtgatctcattaaggaagagttaaccaaaggcaaggctctaggcctatcacacacctacgctaacgtacgcatcaaccatgttataaacctgtggggagctgactttgattctaacgggaaccttaaagctatttatgtaacagactctgatagtaatgcatctattggtatgaagaaatactttgttggtgttaattccgctggaaaagtagctatttctgctaaagaaataaaagaagataatataggtgctcaagtactagggttatttacactttcaacagggcaaaaaagttggaatcagaccaatggcggtggccatcatcaccatcaccactaa

SEQ ID NO: 86 - DNA, 963 bp, Streptococcus pyogenes
atggacgattaccaaaggaatgctacggaagcttatgccaaagaagtaccacatcagatcacttccgtttggaccaaaggagttactcctccagcaaacttcactcaaggtgaagatgtttttcacgctccttatgttgctaaccaaggatggtatgatattaccaaaacattcaatggaaaagacgatcttctttgcggggctgccacagcagggaatatgcttcactggtggttcgatcaaaacaaagaccaaattgaacgttatttggaagagcatccagaaaagcaaaaaataaacttcaaaggcgaacagatgtttgacgtaaaaaaagctatcgacactaaaaaccaccagctagatagtaaattatttgaatattttaaagaaaaagctttcccttatctatctactaaacacctaggagttttccctgatcatgtaattgatatgttcattaacggctaccgccttagtctaactaaccacggtccaacgccagtaaaagaaggtagtaaagatccccgaggtggtatttttgacgccgtatttacaagaggtaaccaaagtaagctattgacaagtcgtcatgattttaaagaaaaaaatctcaaagaaatcagtgatctcattaaggaagagttaaccaaaggcaaggctctaggcctatcacacacctacgctaacgtacgcatcaaccatgttataaacctgtggggagctgactttgattctaacgggaaccttaaagctatttatgtaacagactctgatagtaatgcatctattggtatgaagaaatactttgttggtgttaattccgctggaaaagtagctatttctgctaaagaaataaaagaagataatataggtgctcaagtactagggttatttacactttcaacagggcaaaaaagttggaatcagaccaatggcggtggccatcatcaccatcaccactaa

SEQ ID NO: 87 - protein, 19 aa, Streptococcus pyogenes
SFSANQEIRYSEVTPYHVT

SEQ ID NO: 88 - protein, 19 aa, Streptococcus pyogenes
DYQRNATEAYAKEVPHQIT

SEQ ID NO: 89 - protein, 20 aa, Streptococcus pyogenes
DDYQRNATEAYAKEVPHQIT

SEQ ID NO: 90 - protein, 959 aa, Streptococcus pyogenes
EEKTVQVQKGLPSIDSLHYLSENSKKEFKEELSKAGQESQKVKEILAKAQQADKQAQELAKMKIPEKIPMKPLHGPLYGGYFRTWHDKTSDPTEKDKVNSMGELPKEVDLAFIFHDWTKDYSLFWKELATKHVPKLNKQGTRVIRTIPWRFLAGGDNSGIAEDTSKYPNTPEGNKALAKAIVDEYVYKYNLDGLDVDVEHDSIPKVDKKEDTAGVERSIQVFEEIGKLIGPKGVDKSRLFIMDSTYMADKNPLIERGAPYINLLLVQVYGSQGEKGGWEPVSNRPEKTMEERWQGYSKYIRPEQYMIGFSFYEENAQEGNLWYDINSRKDEDKANGINTDITGTRAERYARWQPKTGGVKGGIFSYAIDRDGVAHQPKKYAKQKEFKDATDNIFHSDYSVSKALKTVMLKDKSYDLIDEKDFPDKALREAVMAQVGTRKGDLERFNGTLRLDNPAIQSLEGLNKFKKLAQLDLIGLSRITKLDRSVLPANMKPGKDTLETVLETYKKDNKEEPATIPPVSLKVSGLTGLKELDLSGFDRETLAGLDAATLTSLEKVDISGNKLDLAPGTENRQIFDTMLSTISNHVGSNEQTVKFDKQKPTGHYPDTYGKTSLRLPVANEKVDLQSQLLFGTVTNQGTLINSEADYKAYQNHKIAGRSFVDSNYHYNNFKVSYENYTVKVTDSTLGTTTDKTLATDKEETYKVDFFSPADKTKAVHTAKVIVGDEKTMMVNLAEGATVIGGSADPVNARKVFDGQLGSETDNISLGWDSKQSIIFKLKEDGLIKHWRFFNDSARNPETTNKPIQEASLQIFNIKDYNLDNLLENPNKFDDEKYWITVDTYSAQGERATAFSNTLNNITSKYWRVVFDTKGDRYSSPVVPELQILGYPLPNADTIMKTVTTAKELSQQKDKFSQKMLDELKIKEMALETSLNSKIFDVTAINANAGVLKDCIEKRQLLKK

SEQ ID NO: 91 - protein, 312 aa, Streptococcus equi ssp. Zooepidemicus
DDYQRNATEAYAKEVPHQITSVWTKGVTPPEQFTQGEDVIHAPYLAHQGWYDITKAFNGKDDLLCGAATAGNMLHWWFDQNKTEIEAYLSKHPEKQKIIFRNQELFDLKAAIDTKDSQTNSQLFNYFRDKAFPNLSARQLGVMPDLVLDMFINGYYLNVFKTQSTDVNRPYQDKDKRGGIFDAVFTRGNQTTLLTARHDLKNKGLNDISTIIKQELTEGRALALSHTYANVSISHVINLWGADFNAEGNLEAIYVTDSDANASIGMKKYFVGINAHGHVAISAKKIEGENIGAQVLGLFTLSSGKDIWQKLS

SEQ ID NO: 92 - protein, 292 aa, Streptococcus equi ssp. Zooepidemicus
SVWTKGVTPPEQFTQGEDVIHAPYLAHQGWYDITKAFNGKDDLLCGAATAGNMLHWWFDQNKTEIEAYLSKHPEKQKIIFRNQELFDLKAAIDTKDSQTNSQLFNYFRDKAFPNLSARQLGVMPDLVLDMFINGYYLNVFKTQSTDVNRPYQDKDKRGGIFDAVFTRGNQTTLLTARHDLKNKGLNDISTIIKQELTEGRALALSHTYANVSISHVINLWGADFNAEGNLEAIYVTDSDANASIGMKKYFVGINAHGHVAISAKKIEGENIGAQVLGLFTLSSGKDIWQKLS